European Patent Specification EP 3 521 424 B1, published April 16, 2025. Title: Method for designing primers used for multiplex PCR. Applicant: FUJI FILM CORP. The sequence listing filed with the application follows.

SEQUENCE LISTING (64 sequences)

SEQ ID NO: 1 - DNA, 20 bp, Artificial Sequence
  chr13.20763642-F
tagccggatgtgggagatgg

SEQ ID NO: 2 - DNA, 20 bp, Artificial Sequence
  chr13.20763642-R
ccagcattggaaagatctgg

SEQ ID NO: 3 - DNA, 20 bp, Artificial Sequence
  chr13.24798120-F
ccgtgtgtgagattctcgtg

SEQ ID NO: 4 - DNA, 20 bp, Artificial Sequence
  chr13.24798120-R
actgctcagggtcctctgtg

SEQ ID NO: 5 - DNA, 20 bp, Artificial Sequence
  chr13.25265103-F
ggcctagaggacgatgcttg

SEQ ID NO: 6 - DNA, 20 bp, Artificial Sequence
  chr13.25265103-R
tgttgataaccatgccggtg

SEQ ID NO: 7 - DNA, 20 bp, Artificial Sequence
  chr13.27845654-F
ccttcactccccccagtttg

SEQ ID NO: 8 - DNA, 20 bp, Artificial Sequence
  chr13.27845654-R
gcataaaagcagggagcgtg

SEQ ID NO: 9 - DNA, 20 bp, Artificial Sequence
  chr13.36385031-F
gagccacgtatgttggggtg

SEQ ID NO: 10 - DNA, 20 bp, Artificial Sequence
  chr13.36385031-R
aaagggcttttgagctcttg

SEQ ID NO: 11 - DNA, 20 bp, Artificial Sequence
  chr13.36743177-F
aaaccatgccaactcttttg

SEQ ID NO: 12 - DNA, 20 bp, Artificial Sequence
  chr13.36743177-R
tctttgcagcaacagttttg

SEQ ID NO: 13 - DNA, 20 bp, Artificial Sequence
  chr13.36801415-F
agatcacaatcctgggggtg

SEQ ID NO: 14 - DNA, 20 bp, Artificial Sequence
  chr13.36801415-R
gggtttcagtgctgcaggtg

SEQ ID NO: 15 - DNA, 20 bp, Artificial Sequence
  chr13.36886469-F
gctgcacattccaatccttg

SEQ ID NO: 16 - DNA, 20 bp, Artificial Sequence
  chr13.36886469-R
agatgggaaatctcctctgg

SEQ ID NO: 17 - DNA, 20 bp, Artificial Sequence
  chr13.46946157-F
tctcaggatatggggaggtg

SEQ ID NO: 18 - DNA, 20 bp, Artificial Sequence
  chr13.46946157-R
ggataccacagactccgttg

SEQ ID NO: 19 - DNA, 20 bp, Artificial Sequence
  chr13.52544805-F
atgcacaggtcatgcctttg

SEQ ID NO: 20 - DNA, 20 bp, Artificial Sequence
  chr13.52544805-R
atggtgcaaactacagatgg

SEQ ID NO: 21 - DNA, 20 bp, Artificial Sequence
  chr13.53608479-F
aaagctcagattccagcttg

SEQ ID NO: 22 - DNA, 20 bp, Artificial Sequence
  chr13.53608479-R
ctctgtccacgggaaaggtg

SEQ ID NO: 23 - DNA, 20 bp, Artificial Sequence
  chr13.67800935-F
gtaacaatcacagccgcttg

SEQ ID NO: 24 - DNA, 20 bp, Artificial Sequence
  chr13.67800935-R
accgaatgcctccttctttg

SEQ ID NO: 25 - DNA, 20 bp, Artificial Sequence
  chr13.95858978-F
cgaggagcacgtaggtggtg

SEQ ID NO: 26 - DNA, 20 bp, Artificial Sequence
  chr13.95858978-R
tgagccactttatctggttg

SEQ ID NO: 27 - DNA, 20 bp, Artificial Sequence
  chr13.102366825-F
cattgtgggaagtgcatttg

SEQ ID NO: 28 - DNA, 20 bp, Artificial Sequence
  chr13.102366825-R
tgcatgacgagtgtctcttg

SEQ ID NO: 29 - DNA, 20 bp, Artificial Sequence
  chr13.103396716-F
ttcagatgacatgaggctgg

SEQ ID NO: 30 - DNA, 20 bp, Artificial Sequence
  chr13.103396716-R
acagggaaatcaaagattgg

SEQ ID NO: 31 - DNA, 20 bp, Artificial Sequence
  chr13.103397937-F
cagcaccagccctgatattg

SEQ ID NO: 32 - DNA, 20 bp, Artificial Sequence
  chr13.103397937-R
aaagagacagcgatttttgg

SEQ ID NO: 33 - DNA, 20 bp, Artificial Sequence
  chr13.111098226-F
gccattgcagtccctttttg

SEQ ID NO: 34 - DNA, 20 bp, Artificial Sequence
  chr13.111098226-R
tgggcgagacaccataagtg

SEQ ID NO: 35 - DNA, 20 bp, Artificial Sequence
  chr13.20763380-F
cttcgatgcggaccttctgg

SEQ ID NO: 36 - DNA, 20 bp, Artificial Sequence
  chr13.20763380-R
tctcccacatccggctatgg

SEQ ID NO: 37 - DNA, 20 bp, Artificial Sequence
  chr13.21086599-F
cccacttccattccttctgg

SEQ ID NO: 38 - DNA, 20 bp, Artificial Sequence
  chr13.21086599-R
cccttcagtggagtcattgg

SEQ ID NO: 39 - DNA, 20 bp, Artificial Sequence
  chr13.21205192-F
tttccccgaccataagcttg

SEQ ID NO: 40 - DNA, 20 bp, Artificial Sequence
  chr13.21205192-R
atacagggctgagagattgg

SEQ ID NO: 41 - DNA, 20 bp, Artificial Sequence
  chr13.21383364-F
attcctacactggccagttg

SEQ ID NO: 42 - DNA, 20 bp, Artificial Sequence
  chr13.21383364-R
agccacagaagtgcacgttg

SEQ ID NO: 43 - DNA, 20 bp, Artificial Sequence
  chr13.21620085-F
tgataaggtccgaactttgg

SEQ ID NO: 44 - DNA, 20 bp, Artificial Sequence
  chr13.21620085-R
gcgactgcaagagattcgtg

SEQ ID NO: 45 - DNA, 20 bp, Artificial Sequence
  chr13.23898664-F
gtacctgtctgtggccggtg

SEQ ID NO: 46 - DNA, 20 bp, Artificial Sequence
  chr13.23898664-R
cctcagtctttcacgatgtg

SEQ ID NO: 47 - DNA, 20 bp, Artificial Sequence
  chr13.23908034-F
gagccttcaagatgcttgtg

SEQ ID NO: 48 - DNA, 20 bp, Artificial Sequence
  chr13.23908034-R
ttttccaaatgcccagagtg

SEQ ID NO: 49 - DNA, 20 bp, Artificial Sequence
  chr13.25009099-F
aatccagctcagggaaggtg

SEQ ID NO: 50 - DNA, 20 bp, Artificial Sequence
  chr13.25009099-R
atcccacagtcggcgtcttg

SEQ ID NO: 51 - DNA, 20 bp, Artificial Sequence
  chr13.25029218-F
ccaaagcgcactcacctgtg

SEQ ID NO: 52 - DNA, 20 bp, Artificial Sequence
  chr13.25029218-R
tagccagtgagagcgaagtg

SEQ ID NO: 53 - DNA, 20 bp, Artificial Sequence
  chr13.25265103-F
ggccttgggaatgtggtgtg

SEQ ID NO: 54 - DNA, 20 bp, Artificial Sequence
  chr13.25265103-R
ggcaatatggccaatgatgg

SEQ ID NO: 55 - DNA, 20 bp, Artificial Sequence
  chr13.25266932-F
tgctggacagtgactcatgg

SEQ ID NO: 56 - DNA, 20 bp, Artificial Sequence
  chr13.25266932-R
cattttcctgtcctggcttg

SEQ ID NO: 57 - DNA, 20 bp, Artificial Sequence
  chr13.28610183-F
ttcttccaggtccaagatgg

SEQ ID NO: 58 - DNA, 20 bp, Artificial Sequence
  chr13.28610183-R
ttggcttcacaaagtattgg

SEQ ID NO: 59 - DNA, 20 bp, Artificial Sequence
  chr13.28624294-F
cctgcccagttcatttctgg

SEQ ID NO: 60 - DNA, 20 bp, Artificial Sequence
  chr13.28624294-R
tcctcttgagcattcatttg

SEQ ID NO: 61 - DNA, 20 bp, Artificial Sequence
  chr13.26043182-F
cctggcggttgacttctttg

SEQ ID NO: 62 - DNA, 20 bp, Artificial Sequence
  chr13.26043182-R
aatttgttgagatgcggttg

SEQ ID NO: 63 - DNA, 20 bp, Artificial Sequence
  chr13.28367956-F
agaagcaggtgaagatctgg

SEQ ID NO: 64 - DNA, 20 bp, Artificial Sequence
  chr13.28367956-R
cgtcatcctcggagcacttg